European Patent Application EP 4 292 610 A1, published December 20, 2023. Title: Variant antibodies that bind gamma-delta T cell receptors. Applicant: LAVA Therapeutics. The sequence listing filed with the application follows.

SEQUENCE LISTING (36 sequences)

SEQ ID NO: 1 - protein, 5 aa, Artificial Sequence
  antibody sequence
  MISC_FEATURE (5)..(5): X is S or G
NYAMX

SEQ ID NO: 2 - protein, 17 aa, Artificial Sequence
  antibody sequence
AISWSGGSTSYADSVKG

SEQ ID NO: 3 - protein, 21 aa, Artificial Sequence
  antibody sequence
  MISC_FEATURE (7)..(7): X can be any amino acid
  MISC_FEATURE (11)..(11): X is not R
QFSGADXGFGXLGIRGYEYDY

SEQ ID NO: 4 - protein, 130 aa, Artificial Sequence
  antibody sequence
  MISC_FEATURE (35)..(35): X is S or G
  MISC_FEATURE (105)..(105): X can be any amino acid
  MISC_FEATURE (109)..(109): X is not R
EVQLLESGGGSVQPGGSLRLSCAASGRPFSNYAMXWFRQAPGKEREFVSAISWSGGSTSYADSVKGRFTISRDNSKNTLYLQMNSLRAEDTAVYYCAAQFSGADXGFGXLGIRGYEYDYWGQGTQVTVSS

SEQ ID NO: 5 - protein, 5 aa, Artificial Sequence
  antibody sequence
SYGMG

SEQ ID NO: 6 - protein, 17 aa, Artificial Sequence
  antibody sequence
GISWRGDSTGYADSVKG

SEQ ID NO: 7 - protein, 15 aa, Artificial Sequence
  antibody sequence
AAGSAWYGTLYEYDY

SEQ ID NO: 8 - protein, 124 aa, Artificial Sequence
  antibody sequence
EVQLVESGGGSVQPGGSLRLSCAASGRTSRSYGMGWFRQAPGKEREFVSGISWRGDSTGYADSVKGRFTISRDNAKNTVDLQMNSLRAEDTAVYYCAAAAGSAWYGTLYEYDYWGQGTLVTVSS

SEQ ID NO: 9 - protein, 10 aa, Artificial Sequence
  antibody sequence
  MISC_FEATURE (10)..(10): X is G or S
GRTASSYVMX

SEQ ID NO: 10 - protein, 17 aa, Artificial Sequence
  antibody sequence
  MISC_FEATURE (12)..(12): X is A or T
VINWNGDSTYYXDSVKG

SEQ ID NO: 11 - protein, 22 aa, Artificial Sequence
  antibody sequence
  MISC_FEATURE (11)..(11): X is Y or F
DTRREWYRDGXWGPPARYEYDY

SEQ ID NO: 12 - protein, 131 aa, Artificial Sequence
  antibody sequence
EVQLVESGGGLVQAGGSLRLSCAASGRTASSYVMGWFRQAPGKEREFVAVINWNGDSTYYTDSVKGRFAISRDNAKNTVYLQMNSLKPEDTAVYYCAADTRREWYRDGYWGPPARYEYDYRGQGTQVTVSS

SEQ ID NO: 13 - protein, 5 aa, Artificial Sequence
  antibody sequence
GGGGS

SEQ ID NO: 14 - protein, 14 aa, Artificial Sequence
  antibody sequence
AAASDKTHTCPPCP

SEQ ID NO: 15 - protein, 231 aa, Artificial Sequence
  antibody sequence
  MISC_FEATURE (231)..(231): X is K or absent
AAASDKTHTCPPCPAPEFEGGPSVFLFPPKPKDTLMISRTPEVTCVVVDVSHEDPEVKFNWYVDGVEVHNAKTKPREEQYNSTYRVVSVLTVLHQDWLNGKEYKCKVSNKALPAPIEKTISKAKGQPREPQVYTLPPSRDELTKNQVSLWCLVKGFYPSDIAVEWESNGQPENNYKTTPPVLDSDGSFFLYSKLTVDKSRWQQGNVFSCSVMHEALHNHYTQKSLSLSPGX

SEQ ID NO: 16 - protein, 231 aa, Artificial Sequence
  antibody sequence
  MISC_FEATURE (231)..(231): X is K or absent
AAASDKTHTCPPCPAPEFEGGPSVFLFPPKPKDTLMISRTPEVTCVVVDVSHEDPEVKFNWYVDGVEVHNAKTKPREEQYNSTYRVVSVLTVLHQDWLNGKEYKCKVSNKALPAPIEKTISKAKGQPREPQVYTLPPSRDELTKNQVSLSCAVKGFYPSDIAVEWESNGQPENNYKTTPPVLDSDGSFFLVSKLTVDKSRWQQGNVFSCSVMHEALHNHYTQKSLSLSPGX

SEQ ID NO: 17 - protein, 130 aa, Artificial Sequence
  antibody sequence
EVQLVESGGGLVQAGGSLRLSCAASGRPFSNYAMGWFRQAPGKEREFVAAISWSGGSTSYADSVKGRFTISRDNAKNTVYLQMNSPKPEDTAIYYCAAQFSGADYGFGRLGIRGYEYDYWGQGTQVTVSS

SEQ ID NO: 18 - protein, 130 aa, Artificial Sequence
  antibody sequence
EVQLLESGGGSVQPGGSLRLSCAASGRPFSNYAMSWFRQAPGKEREFVSAISWSGGSTSYADSVKGRFTISRDNSKNTLYLQMNSLRAEDTAVYYCAAQFSGADYGFGRLGIRGYEYDYWGQGTQVTVSS

SEQ ID NO: 19 - protein, 21 aa, Artificial Sequence
  antibody sequence
QFSGADYGFGRLGIRGYEYDY

SEQ ID NO: 20 - protein, 355 aa, Artificial Sequence
  antibody sequence
  MISC_FEATURE (355)..(355): X is K or absent
EVQLVESGGGSVQPGGSLRLSCAASGRTSRSYGMGWFRQAPGKEREFVSGISWRGDSTGYADSVKGRFTISRDNAKNTVDLQMNSLRAEDTAVYYCAAAAGSAWYGTLYEYDYWGQGTLVTVSSAAASDKTHTCPPCPAPEFEGGPSVFLFPPKPKDTLMISRTPEVTCVVVDVSHEDPEVKFNWYVDGVEVHNAKTKPREEQYNSTYRVVSVLTVLHQDWLNGKEYKCKVSNKALPAPIEKTISKAKGQPREPQVYTLPPSRDELTKNQVSLSCAVKGFYPSDIAVEWESNGQPENNYKTTPPVLDSDGSFFLVSKLTVDKSRWQQGNVFSCSVMHEALHNHYTQKSLSLSPGX

SEQ ID NO: 21 - protein, 362 aa, Artificial Sequence
  antibody sequence
  MISC_FEATURE (361)..(361): X is K or absent
  misc_feature (362)..(362): Xaa can be any naturally occurring amino acid
EVQLVESGGGLVQAGGSLRLSCAASGRTASSYVMGWFRQAPGKEREFVAVINWNGDSTYYTDSVKGRFAISRDNAKNTVYLQMNSLKPEDTAVYYCAADTRREWYRDGYWGPPARYEYDYRGQGTQVTVSSAAASDKTHTCPPCPAPEFEGGPSVFLFPPKPKDTLMISRTPEVTCVVVDVSHEDPEVKFNWYVDGVEVHNAKTKPREEQYNSTYRVVSVLTVLHQDWLNGKEYKCKVSNKALPAPIEKTISKAKGQPREPQVYTLPPSRDELTKNQVSLSCAVKGFYPSDIAVEWESNGQPENNYKTTPPVLDSDGSFFLVSKLTVDKSRWQQGNVFSCSVMHEALHNHYTQKSLSLSPGX

SEQ ID NO: 22 - protein, 361 aa, Artificial Sequence
  antibody sequence
  MISC_FEATURE (361)..(361): X is K or absent
EVQLLESGGGSVQPGGSLRLSCAASGRPFSNYAMSWFRQAPGKEREFVSAISWSGGSTSYADSVKGRFTISRDNSKNTLYLQMNSLRAEDTAVYYCAAQFSGADFGFGALGIRGYEYDYWGQGTQVTVSSAAASDKTHTCPPCPAPEFEGGPSVFLFPPKPKDTLMISRTPEVTCVVVDVSHEDPEVKFNWYVDGVEVHNAKTKPREEQYNSTYRVVSVLTVLHQDWLNGKEYKCKVSNKALPAPIEKTISKAKGQPREPQVYTLPPSRDELTKNQVSLWCLVKGFYPSDIAVEWESNGQPENNYKTTPPVLDSDGSFFLYSKLTVDKSRWQQGNVFSCSVMHEALHNHYTQKSLSLSPGX

SEQ ID NO: 23 - protein, 361 aa, Artificial Sequence
  antibody sequence
  MISC_FEATURE (361)..(361): X is K or absent
EVQLLESGGGSVQPGGSLRLSCAASGRPFSNYAMSWFRQAPGKEREFVSAISWSGGSTSYADSVKGRFTISRDNSKNTLYLQMNSLRAEDTAVYYCAAQFSGADSGFGALGIRGYEYDYWGQGTQVTVSSAAASDKTHTCPPCPAPEFEGGPSVFLFPPKPKDTLMISRTPEVTCVVVDVSHEDPEVKFNWYVDGVEVHNAKTKPREEQYNSTYRVVSVLTVLHQDWLNGKEYKCKVSNKALPAPIEKTISKAKGQPREPQVYTLPPSRDELTKNQVSLWCLVKGFYPSDIAVEWESNGQPENNYKTTPPVLDSDGSFFLYSKLTVDKSRWQQGNVFSCSVMHEALHNHYTQKSLSLSPGX

SEQ ID NO: 24 - protein, 361 aa, Artificial Sequence
  antibody sequence
  MISC_FEATURE (361)..(361): X is K or absent
EVQLLESGGGSVQPGGSLRLSCAASGRPFSNYAMSWFRQAPGKEREFVSAISWSGGSTSYADSVKGRFTISRDNSKNTLYLQMNSLRAEDTAVYYCAAQFSGADFGFGKLGIRGYEYDYWGQGTQVTVSSAAASDKTHTCPPCPAPEFEGGPSVFLFPPKPKDTLMISRTPEVTCVVVDVSHEDPEVKFNWYVDGVEVHNAKTKPREEQYNSTYRVVSVLTVLHQDWLNGKEYKCKVSNKALPAPIEKTISKAKGQPREPQVYTLPPSRDELTKNQVSLWCLVKGFYPSDIAVEWESNGQPENNYKTTPPVLDSDGSFFLYSKLTVDKSRWQQGNVFSCSVMHEALHNHYTQKSLSLSPGX

SEQ ID NO: 25 - protein, 361 aa, Artificial Sequence
  antibody sequence
  MISC_FEATURE (361)..(361): X is K or absent
EVQLLESGGGSVQPGGSLRLSCAASGRPFSNYAMSWFRQAPGKEREFVSAISWSGGSTSYADSVKGRFTISRDNSKNTLYLQMNSLRAEDTAVYYCAAQFSGADSGFGKLGIRGYEYDYWGQGTQVTVSSAAASDKTHTCPPCPAPEFEGGPSVFLFPPKPKDTLMISRTPEVTCVVVDVSHEDPEVKFNWYVDGVEVHNAKTKPREEQYNSTYRVVSVLTVLHQDWLNGKEYKCKVSNKALPAPIEKTISKAKGQPREPQVYTLPPSRDELTKNQVSLWCLVKGFYPSDIAVEWESNGQPENNYKTTPPVLDSDGSFFLYSKLTVDKSRWQQGNVFSCSVMHEALHNHYTQKSLSLSPGX

SEQ ID NO: 26 - protein, 131 aa, artificial sequence
  antibody sequence
EVQLVESGGGLVQPGGSLRLSCAASGRTASSYVMGWFRQAPGKEREFVSVINWNGDSTYYADSVKGRFTISRDNSKNTLYLQMNSLRAEDTAVYYCAADTRREWYRDGYWGPPARYEYDYRGQGTQVTVSS

SEQ ID NO: 27 - protein, 131 aa, artificial sequence
  antibody sequence
EVQLVESGGGLVQPGGSLRLSCAASGRTASSYVMGWVRQAPGKEREWVSVINWNGDSTYYADSVKGRFTISRDNSKNTLYLQMNSLRAEDTAVYYCAADTRREWYRDGYWGPPARYEYDYRGQGTLVTVSS

SEQ ID NO: 28 - protein, 131 aa, artificial sequence
  antibody sequence
EVQLVESGGGLVQPGGSLRLSCAASGRTASSYVMSWFRQAPGKEREWVAVINWNGDSTYYADSVKGRFTISRDNSKNTVYLQMNSLRAEDTAVYYCAADTRREWYRDGYWGPPARYEYDYRGQGTLVTVSS

SEQ ID NO: 29 - protein, 131 aa, artificial sequence
  antibody sequence
EVQLVESGGGVVQPGGSLRLSCAASGRTASSYVMSWFRQAPGKEREWVAVINWNGDSTYYADSVKGRFTISRDNSKNTLYLQMNSLRAEDTAVYYCAADTRREWYRDGYWGPPARYEYDYRGQGTTVTVSS

SEQ ID NO: 30 - protein, 131 aa, artificial sequence
  antibody sequence
EVQLVESGGGLVQPGGSLRLSCAASGRTASSYVMSWFRQAPGKEREFVAVINWNGDSTYYADSVKGRFTISRDNSKNTVYLQMNSLRAEDTAVYYCAADTRREWYRDGYWGPPARYEYDYRGQGTLVTVSS

SEQ ID NO: 31 - protein, 131 aa, artificial sequence
  antibody sequence
EVQLVESGGGLVQPGGSLRLSCAASGRTASSYVMGWVRQAPGKGLEWVSVINWNGDSTYYADSVKGRFTISRDNSKNTLYLQMNSLRAEDTAVYYCAADTRREWYRDGYWGPPARYEYDYRGQGTLVTVSS

SEQ ID NO: 32 - protein, 131 aa, artificial sequence
  antibody sequence
EVQLVESGGGLVQPGGSLRLSCAASGRTASSYVMSWVRQAPGKGLEWVSVINWNGDSTYYADSVKGRFTISRDNSKNTLYLQMNSLRAEDTAVYYCAADTRREWYRDGYWGPPARYEYDYRGQGTLVTVSS

SEQ ID NO: 33 - protein, 131 aa, artificial sequence
  antibody sequence
EVQLVESGGGLVQPGGSLRLSCAASGRTASSYVMSWFRQAPGKGLEWVAVINWNGDSTYYADSVKGRFTISRDNSKNTVYLQMNSLRAEDTAVYYCAADTRREWYRDGYWGPPARYEYDYRGQGTLVTVSS

SEQ ID NO: 34 - protein, 131 aa, artificial sequence
  antibody sequence
EVQLVESGGGLVQAGGSLRLSCAASGRTASSYVMGWFRQAPGKEREWVAVINWNGDSTYYTDSVKGRFAISRDNAKNTVYLQMNSLRAEDTAVYYCAADTRREWYRDGYWGPPARYEYDYRGQGTQVTVSS

SEQ ID NO: 35 - protein, 131 aa, artificial sequence
  antibody sequence
EVQLVESGGGLVQPGGSLRLSCAASGRTASSYVMGWFRQAPGKEREFVSVINWNGDSTYYADSVKGRFTISRDNSKNTLYLQMNSLRAEDTAVYYCAADTRREWYRDGFWGPPARYEYDYRGQGTQVTVSS

SEQ ID NO: 36 - protein, 17 aa, artificial sequence
  antibody sequence
QFSGADFGFGAGYEYDY